European Patent Application EP 4 759 319 A1, published June 17, 2026. Title: TREATMENT OF TENDINOPATHY USING PLATELETS PRODUCED FROM ADIPOSE-DERIVED MESENCHYMAL STEM CELL LINE. Applicant: 慶應義塾. The sequence listing filed with the application follows.

SEQUENCE LISTING (12 sequences)

SEQ ID NO: 1 - DNA, 21 bp, synthetic construct
  source 1..21: mol_type = other DNA
tctctccgcaagagacttcca

SEQ ID NO: 2 - DNA, 21 bp, synthetic construct
  source 1..21: mol_type = other DNA
ggtctgttgtgggtggtatcc

SEQ ID NO: 3 - DNA, 19 bp, synthetic construct
  source 1..19: mol_type = other DNA
tgtgatgttcccattagac

SEQ ID NO: 4 - DNA, 19 bp, synthetic construct
  source 1..19: mol_type = other DNA
aataccacttgttggctta

SEQ ID NO: 5 - DNA, 23 bp, synthetic construct
  source 1..23: mol_type = other DNA
gcgtagcctacatggaccaacag

SEQ ID NO: 6 - DNA, 23 bp, synthetic construct
  source 1..23: mol_type = other DNA
aagttccggtgtgactcgtgcag

SEQ ID NO: 7 - DNA, 23 bp, synthetic construct
  source 1..23: mol_type = other DNA
tcgggatctgtcctctgtgatga

SEQ ID NO: 8 - DNA, 23 bp, synthetic construct
  source 1..23: mol_type = other DNA
caggaatgacaggagcaggtgta

SEQ ID NO: 9 - DNA, 25 bp, synthetic construct
  source 1..25: mol_type = other DNA
agcaaccagagaaagttgagcaaag

SEQ ID NO: 10 - DNA, 22 bp, synthetic construct
  source 1..22: mol_type = other DNA
ttccaccttcactagtggcatc

SEQ ID NO: 11 - DNA, 22 bp, synthetic construct
  source 1..22: mol_type = other DNA
tgatggaggtggatggatcgtt

SEQ ID NO: 12 - DNA, 23 bp, synthetic construct
  source 1..23: mol_type = other DNA
ctcaggttatccagtccaagcca